European Patent Specification EP 4 456 713 B1, published November 12, 2025. Title: PRODUCTS AND METHODS FOR IMPROVING PLANT GROWTH FEATURES. Applicant: Aphea.Bio NV. The sequence listing filed with the application follows.

SEQUENCE LISTING (3 sequences)

SEQ ID NO: 1 - DNA, 1544 bp, Stenotrophomonas rhizophila
  source 1..1544: mol_type = genomic DNA
gtgaagagtttgatcctggctcagagtgaacgctggcggtaggcctaacacatgcaagtcgaacggcagcacagtaagagcttgctcttatgggtggcgagtggcggacgggtgaggaatacatcggaatctaccttttcgtgggggataacgtagggaaacttacgctaataccgcatacgaccttcgggtgaaagcaggggaccttcgggccttgcgcggatagatgagccgatgtcggattagctagttggcggggtaaaggcccaccaaggcgacgatccgtagctggtctgagaggatgatcagccacactggaactgagacacggtccagactcctacgggaggcagcagtggggaatattggacaatgggcgcaagcctgatccagccataccgcgtgggtgaagaaggccttcgggttgtaaagcccttttgttgggaaagaaaagcagtcggctaatacccggttgttctgacggtacccaaagaataagcaccggctaacttcgtgccagcagccgcggtaatacgaagggtgcaagcgttactcggaattactgggcgtaaagcgtgcgtaggtggttgtttaagtctgttgtgaaagccctgggctcaacctgggaattgcagtggatactgggcgactagagtgtggtagagggtagtggaattcccggtgtagcagtgaaatgcgtagagatcgggaggaacatccatggcgaaggcagctacctggaccaacactgacactgaggcacgaaagcgtggggagcaaacaggattagataccctggtagtccacgccctaaacgatgcgaactggatgttgggtgcaatttggcacgcagtatcgaagctaacgcgttaagttcgccgcctggggagtacggtcgcaagactgaaactcaaaggaattgacgggggcccgcacaagcggtggagtatgtggtttaattcgatgcaacgcgaagaaccttacctggtcttgacatgtcgagaactttccagagatggattggtgccttcgggaactcgaacacaggtgctgcatggctgtcgtcagctcgtgtcgtgagatgttgggttaagtcccgcaacgagcgcaacccttgtccttagttgccagcacgtaatggtgggaactctaaggagaccgccggtgacaaaccggaggaaggtggggatgacgtcaagtcatcatggcccttacgaccagggctacacacgtactacaatggtagggacagagggctgcaaacccgcgagggcaagccaatcccagaaaccctatctcagtccggattggagtctgcaactcgactccatgaagtcggaatcgctagtaatcgcagatcagcattgctgcggtgaatacgttcccgggccttgtacacaccgcccgtcacaccatgggagtttgttgcaccagaagcaggtagcttaaccttcgggagggcgcttgccacggtgtggccgatgactggggtgaagtcgtaacaaggtagccgtatcggaaggtgcggctggatcacctccttt

SEQ ID NO: 2 - DNA, 20 bp, synthetic construct
  misc_feature 1..20: note = Forward primer 27F
  source 1..20: mol_type = other DNA
agagtttgatcctggctcag

SEQ ID NO: 3 - DNA, 19 bp, synthetic construct
  misc_feature 1..19: note = Reverse primer 1492R
  source 1..19: mol_type = other DNA
ggttaccttgttacgactt